European Patent Specification EP 4 072 584 B1, published January 28, 2026. Title: ANTI-LY6G6D ANTIBODIES AND METHODS OF USE. Applicant: Genentech, Inc. The sequence listing filed with the application follows.

SEQUENCE LISTING (147 sequences)

SEQ ID NO: 1 - protein, 11 aa, Artificial Sequence
  Synthetic Construct
QASESITRYLN

SEQ ID NO: 2 - protein, 7 aa, Artificial Sequence
  Synthetic Construct
DASKLPS

SEQ ID NO: 3 - protein, 13 aa, Artificial Sequence
  Synthetic Construct
QSTSFRGRSYQNT

SEQ ID NO: 4 - protein, 5 aa, Artificial Sequence
  Synthetic Construct
NNAMI

SEQ ID NO: 5 - protein, 17 aa, Artificial Sequence
  Synthetic Construct
ALSFADNTAYYATWASG

SEQ ID NO: 6 - protein, 3 aa, Artificial Sequence
  Synthetic Construct
GDL

SEQ ID NO: 7 - protein, 442 aa, Artificial Sequence
  Synthetic Construct
EVQLLESGGGLVQPGGSLRLSCAASGFDFVNNAMIWVREAPGKGLEWVSALSFADNTAYYATWASGRFTISRDSSKTTVYLQMNSLRAEDTAVYYCMRGDLWGPGTLVTVSSASTKGPSVFPLAPSSKSTSGGTAALGCLVKDYFPEPVTVSWNSGALTSGVHTFPAVLQSSGLYSLKSVVTVPSSSLGTQTYICNVNHKPSNTKVDKKVEPKSCDKTHTCPPCPAPELLGGPSVFLFPPKPKDTLMISRTPEVTCVVVDVSHEDPEVKFNWYVDGVEVHNAKTKPREEQYGSTYRVVSVLTVLHQDWLNGKEYKCKVSNKALPAPIEKTISKAKGQPREPQVYTLPPSREEMTKNQVSLWCLVKGFYPSDIAVEWESNGQPENNYKTTPPVLDSDGSFFLYSKLTVDKSRWQQGNVFSCSVMHEALHNHYTQKSLSLSPGK

SEQ ID NO: 8 - protein, 442 aa, Artificial Sequence
  Synthetic Construct
EVQLLESGGGLVQPGGSLRLSCAASGFDFVNNAMIWVREAPGKGLEWVSALSFADNTAYYATWASGRFTISRDSSKTTVYLQMNSLRAEDTAVYYCMRGDLWGPGTLVTVSSASTKGPSVFPLAPSSKSTSGGTAALGCLVKDYFPEPVTVSWNSGALTSGVHTFPAVLQSSGLYSLKSVVTVPSSSLGTQTYICNVNHKPSNTKVDKKVEPKSCDKTHTCPPCPAPELLGGPSVFLFPPKPKDTLMISRTPEVTCVVVDVSHEDPEVKFNWYVDGVEVHNAKTKPREEQYGSTYRVVSVLTVLHQDWLNGKEYKCKVSNKALPAPIEKTISKAKGQPREPQVYTLPPSREEMTKNQVSLSCAVKGFYPSDIAVEWESNGQPENNYKTTPPVLDSDGSFFLVSKLTVDKSRWQQGNVFSCSVMHEALHNHYTQKSLSLSPGK

SEQ ID NO: 9 - protein, 218 aa, Artificial Sequence
  Synthetic Construct
DIQMTQSPSTLSASVGDRVTITCQASESITRYLNWYQKKPGKAPKLLIYDASKLPSGVPSRFSGSGSGTEFTLTISSLQPDDFATYYCQSTSFRGRSYQNTFGGGTKVEIKRTVAAPSVFIFPPSDEQLKSGTASVECLLNNFYPREAKVQWKVDNALQSGNSQESVTEQDSKDSTYSLSSTLTLSKADYEKHKVYACEVTHQGLSSPVTKSFNRGEC

SEQ ID NO: 10 - protein, 112 aa, Artificial Sequence
  Synthetic Construct
EVQLLESGGGLVQPGGSLRLSCAASGFDFVNNAMIWVREAPGKGLEWVSALSFADNTAYYATWASGRFTISRDSSKTTVYLQMNSLRAEDTAVYYCMRGDLWGPGTLVTVSS

SEQ ID NO: 11 - protein, 111 aa, Artificial Sequence
  Synthetic Construct
DIQMTQSPSTLSASVGDRVTITCQASESITRYLNWYQKKPGKAPKLLIYDASKLPSGVPSRFSGSGSGTEFTLTISSLQPDDFATYYCQSTSFRGRSYQNTFGGGTKVEIK

SEQ ID NO: 12 - protein, 17 aa, Artificial Sequence
  Synthetic Construct
KSSQSLLNSRTRKNYLA

SEQ ID NO: 13 - protein, 7 aa, Artificial Sequence
  Synthetic Construct
WASTRES

SEQ ID NO: 14 - protein, 8 aa, Artificial Sequence
  Synthetic Construct
TQSFILRT

SEQ ID NO: 15 - protein, 5 aa, Artificial Sequence
  Synthetic Construct
SYYIH

SEQ ID NO: 16 - protein, 17 aa, Artificial Sequence
  Synthetic Construct
WIYPENDNTKYNEKFKD

SEQ ID NO: 17 - protein, 10 aa, Artificial Sequence
  Synthetic Construct
DGYSRYYFDY

SEQ ID NO: 18 - protein, 449 aa, Artificial Sequence
  Synthetic Construct
EVQLVQSGAEVKKPGASVKVSCKASGFTFTSYYIHWVRKAPGQGLEWIGWIYPENDNTKYNEKFKDRVTITADTSTSTAYLELSSLRSEDTAVYYCARDGYSRYYFDYWGQGTLVTVSSASTKGPSVFPLAPSSKSTSGGTAALGCLVKDYFPEPVTVSWNSGALTSGVHTFPAVLQSSGLYSLESVVTVPSSSLGTQTYICNVNHKPSNTKVDKKVEPKSCDKTHTCPPCPAPELLGGPSVFLFPPKPKDTLMISRTPEVTCVVVDVSHEDPEVKFNWYVDGVEVHNAKTKPREEQYGSTYRVVSVLTVLHQDWLNGKEYKCKVSNKALPAPIEKTISKAKGQPREPQVYTLPPSREEMTKNQVSLSCAVKGFYPSDIAVEWESNGQPENNYKTTPPVLDSDGSFFLVSKLTVDKSRWQQGNVFSCSVMHEALHNHYTQKSLSLSPGK

SEQ ID NO: 19 - protein, 219 aa, Artificial Sequence
  Synthetic Construct
DIVMTQSPDSLAVSLGERATINCKSSQSLLNSRTRKNYLAWYQEKPGQPPKLLIYWASTRESGVPDRFSGSGSGTDFTLTISSLQAEDVAVYYCTQSFILRTFGQGTKVEIKRTVAAPSVFIFPPSDEQLKSGTASVKCLLNNFYPREAKVQWKVDNALQSGNSQESVTEQDSKDSTYSLSSTLTLSKADYEKHKVYACEVTHQGLSSPVTKSFNRGEC

SEQ ID NO: 20 - protein, 119 aa, Artificial Sequence
  Synthetic Construct
EVQLVQSGAEVKKPGASVKVSCKASGFTFTSYYIHWVRKAPGQGLEWIGWIYPENDNTKYNEKFKDRVTITADTSTSTAYLELSSLRSEDTAVYYCARDGYSRYYFDYWGQGTLVTVSS

SEQ ID NO: 21 - protein, 112 aa, Artificial Sequence
  Synthetic Construct
DIVMTQSPDSLAVSLGERATINCKSSQSLLNSRTRKNYLAWYQEKPGQPPKLLIYWASTRESGVPDRFSGSGSGTDFTLTISSLQAEDVAVYYCTQSFILRTFGQGTKVEIK

SEQ ID NO: 22 - protein, 112 aa, Artificial Sequence
  Synthetic Construct
EVQLLESGGGLVQPGGSLRLSCAASGFDFVNNAMIWVRQAPGKGLEWVSALSFADNTAYYATWASGRFTISRDSSKTTVYLQMNSLRAEDTAVYYCMRGDLWGPGTLVTVSS

SEQ ID NO: 23 - protein, 111 aa, Artificial Sequence
  Synthetic Construct
DIQMTQSPSTLSASVGDRVTITCQASESITRYLNWYQQKPGKAPKLLIYDASKLPSGVPSRFSGSGSGTEFTLTISSLQPDDFATYYCQSTSFRGRSYQNTFGGGTKVEIK

SEQ ID NO: 24 - protein, 16 aa, Artificial Sequence
  Synthetic Construct
KSSQSLLDSDGRTYLH

SEQ ID NO: 25 - protein, 7 aa, Artificial Sequence
  Synthetic Construct
LVSNLDS

SEQ ID NO: 26 - protein, 9 aa, Artificial Sequence
  Synthetic Construct
WQGTHLPFT

SEQ ID NO: 27 - protein, 5 aa, Artificial Sequence
  Synthetic Construct
SYWIQ

SEQ ID NO: 28 - protein, 18 aa, Artificial Sequence
  Synthetic Construct
EILPGSDNTNYNEKFKGK

SEQ ID NO: 29 - protein, 4 aa, Artificial Sequence
  Synthetic Construct
WFAY

SEQ ID NO: 30 - protein, 443 aa, Artificial Sequence
  Synthetic Construct
QVQLQQSGAELMKPGASVKISCKASGYTFSSYWIQWIKQRPGHGLEWIGEILPGSDNTNYNEKFKGKATFTADTSSSTAYMQLSSLTSEDSAIYYCAKWFAYWGQGTTVTVSAASTKGPSVFPLAPSSKSTSGGTAALGCLVKDYFPEPVTVSWNSGALTSGVHTFPAVLQSSGLYSLSSVVTVPSSSLGTQTYICNVNHKPSNTKVDKKVEPKSCDKTHTCPPCPAPELLGGPSVFLFPPKPKDTLMISRTPEVTCVVVDVSHEDPEVKFNWYVDGVEVHNAKTKPREEQYGSTYRVVSVLTVLHQDWLNGKEYKCKVSNKALPAPIEKTISKAKGQPREPQVYTLPPSREEMTKNQVSLTCLVKGFYPSDIAVEWESNGQPENNYKTTPPVLDSDGSFFLYSKLTVDKSRWQQGNVFSCSVMHEALHNHYTQKSLSLSPGK

SEQ ID NO: 31 - protein, 219 aa, Artificial Sequence
  Synthetic Construct
DIVMTQTPLTLSVTIGHPASISCKSSQSLLDSDGRTYLHWLFQRPGQSPRRLIYLVSNLDSGVPDRFTGSGSGTDFTLKISRVEAEDLGVYYCWQGTHLPFTFGSGTKVEIKRTVAAPSVFIFPPSDEQLKSGTASVVCLLNNFYPREAKVQWKVDNALQSGNSQESVTEQDSKDSTYSLSSTLTLSKADYEKHKVYACEVTHQGLSSPVTKSFNRGEC

SEQ ID NO: 32 - protein, 113 aa, Artificial Sequence
  Synthetic Construct
QVQLQQSGAELMKPGASVKISCKASGYTFSSYWIQWIKQRPGHGLEWIGEILPGSDNTNYNEKFKGKATFTADTSSSTAYMQLSSLTSEDSAIYYCAKWFAYWGQGTTVTVSA

SEQ ID NO: 33 - protein, 112 aa, Artificial Sequence
  Synthetic Construct
DIVMTQTPLTLSVTIGHPASISCKSSQSLLDSDGRTYLHWLFQRPGQSPRRLIYLVSNLDSGVPDRFTGSGSGTDFTLKISRVEAEDLGVYYCWQGTHLPFTFGSGTKVEIK

SEQ ID NO: 34 - protein, 30 aa, Artificial Sequence
  Synthetic Construct
EVQLLESGGGLVQPGGSLRLSCAASGFDFV

SEQ ID NO: 35 - protein, 14 aa, Artificial Sequence
  Synthetic Construct
WVREAPGKGLEWVS

SEQ ID NO: 36 - protein, 32 aa, Artificial Sequence
  Synthetic Construct
RFTISRDSSKTTVYLQMNSLRAEDTAVYYCMR

SEQ ID NO: 37 - protein, 11 aa, Artificial Sequence
  Synthetic Construct
WGPGTLVTVSS

SEQ ID NO: 38 - protein, 23 aa, Artificial Sequence
  Synthetic Construct
DIQMTQSPSTLSASVGDRVTITC

SEQ ID NO: 39 - protein, 15 aa, Artificial Sequence
  Synthetic Construct
WYQKKPGKAPKLLIY

SEQ ID NO: 40 - protein, 32 aa, Artificial Sequence
  Synthetic Construct
GVPSRFSGSGSGTEFTLTISSLQPDDFATYYC

SEQ ID NO: 41 - protein, 10 aa, Artificial Sequence
  Synthetic Construct
FGGGTKVEIK

SEQ ID NO: 42 - protein, 30 aa, Artificial Sequence
  Synthetic Construct
EVQLVQSGAEVKKPGASVKVSCKASGFTFT

SEQ ID NO: 43 - protein, 14 aa, Artificial Sequence
  Synthetic Construct
WVREAPGQGLEWIG

SEQ ID NO: 44 - protein, 32 aa, Artificial Sequence
  Synthetic Construct
RVTITADTSTSTAYLELSSLRSEDTAVYYCAR

SEQ ID NO: 45 - protein, 11 aa, Artificial Sequence
  Synthetic Construct
WGQGTLVTVSS

SEQ ID NO: 46 - protein, 23 aa, Artificial Sequence
  Synthetic Construct
DIVMTQSPDSLAVSLGERATINC

SEQ ID NO: 47 - protein, 15 aa, Artificial Sequence
  Synthetic Construct
WYQQKPGQPPKLLIY

SEQ ID NO: 48 - protein, 32 aa, Artificial Sequence
  Synthetic Construct
GVPDRFSGSGSGTDFTLTISSLQAEDVAVYYC

SEQ ID NO: 49 - protein, 10 aa, Artificial Sequence
  Synthetic Construct
FGQGTKVEIK

SEQ ID NO: 50 - protein, 7 aa, Artificial Sequence
  Synthetic Construct
WASTRKS

SEQ ID NO: 51 - protein, 9 aa, Artificial Sequence
  Synthetic Construct
KQSFILRTF

SEQ ID NO: 52 - protein, 119 aa, Artificial Sequence
  Synthetic Construct
EVQLVQSGAEVKKPGASVKVSCKASGFTFTSYYIHWVRQAPGQGLEWIGWIYPENDNTKYNEKFKDRVTITADTSTSTAYLELSSLRSEDTAVYYCARDGYSRYYFDYWGQGTLVTVSS

SEQ ID NO: 53 - protein, 112 aa, Artificial Sequence
  Synthetic Construct
DIVMTQSPDSLAVSLGERATINCKSSQSLLNSRTRKNYLAWYQQKPGQPPKLLIYWASTRESGVPDRFSGSGSGTDFTLTISSLQAEDVAVYYCTQSFILRTFGQGTKVEIK

SEQ ID NO: 54 - skipped

SEQ ID NO: 55 - protein, 112 aa, Artificial Sequence
  Synthetic Construct
DIVMTQSPDSLAVSLGERATINCKSSQSLLNSRTRKNYLAWYQEKPGQPPKLLIYWASTRKSGVPDRFSGSGSGTDFTLTISSLQAEDVAVYYCKQSFILRTFGQGTKVEIK

SEQ ID NO: 56 - skipped

SEQ ID NO: 57 - protein, 219 aa, Artificial Sequence
  Synthetic Construct
DIVMTQSPDSLAVSLGERATINCKSSQSLLNSRTRKNYLAWYQEKPGQPPKLLIYWASTRKSGVPDRFSGSGSGTDFTLTISSLQAEDVAVYYCKQSFILRTFGQGTKVEIKRTVAAPSVFIFPPSDEQLKSGTASVKCLLNNFYPREAKVQWKVDNALQSGNSQESVTEQDSKDSTYSLSSTLTLSKADYEKHKVYACEVTHQGLSSPVTKSFNRGEC

SEQ ID NO: 58 - protein, 14 aa, Artificial Sequence
  Synthetic Construct
WVRKAPGKGLEWVS

SEQ ID NO: 59 - protein, 112 aa, Artificial Sequence
  Synthetic Construct
EVQLLESGGGLVQPGGSLRLSCAASGFDFVNNAMIWVRKAPGKGLEWVSALSFADNTAYYATWASGRFTISRDSSKTTVYLQMNSLRAEDTAVYYCMRGDLWGPGTLVTVSS

SEQ ID NO: 60 - protein, 111 aa, Artificial Sequence
  Synthetic Construct
DIQMTQSPSTLSASVGDRVTITCQASESITRYLNWYQEKPGKAPKLLIYDASKLPSGVPSRFSGSGSGTEFTLTISSLQPDDFATYYCQSTSFRGRSYQNTFGGGTKVEIK

SEQ ID NO: 61 - protein, 15 aa, Artificial Sequence
  Synthetic Construct
WYQEKPGKAPKLLIY

SEQ ID NO: 62 - protein, 14 aa, Artificial Sequence
  Synthetic Construct
WVRKAPGQGLEWIG

SEQ ID NO: 63 - protein, 15 aa, Artificial Sequence
  Synthetic Construct
WYQQEPGQPPKLLIY

SEQ ID NO: 64 - protein, 442 aa, Artificial Sequence
  Synthetic Construct
EVQLLESGGGLVQPGGSLRLSCAASGFDFVNNAMIWVRKAPGKGLEWVSALSFADNTAYYATWASGRFTISRDSSKTTVYLQMNSLRAEDTAVYYCMRGDLWGPGTLVTVSSASTKGPSVFPLAPSSKSTSGGTAALGCLVKDYFPEPVTVSWNSGALTSGVHTFPAVLQSSGLYSLESVVTVPSSSLGTQTYICNVNHKPSNTKVDKKVEPKSCDKTHTCPPCPAPELLGGPSVFLFPPKPKDTLMISRTPEVTCVVVDVSHEDPEVKFNWYVDGVEVHNAKTKPREEQYGSTYRVVSVLTVLHQDWLNGKEYKCKVSNKALPAPIEKTISKAKGQPREPQVYTLPPSREEMTKNQVSLWCLVKGFYPSDIAVEWESNGQPENNYKTTPPVLDSDGSFFLYSKLTVDKSRWQQGNVFSCSVMHEALHNHYTQKSLSLSPGK

SEQ ID NO: 65 - protein, 218 aa, Artificial Sequence
  Synthetic Construct
DIQMTQSPSTLSASVGDRVTITCQASESITRYLNWYQEKPGKAPKLLIYDASKLPSGVPSRFSGSGSGTEFTLTISSLQPDDFATYYCQSTSFRGRSYQNTFGGGTKVEIKRTVAAPSVFIFPPSDEQLKSGTASVKCLLNNFYPREAKVQWKVDNALQSGNSQESVTEQDSKDSTYSLSSTLTLSKADYEKHKVYACEVTHQGLSSPVTKSFNRGEC

SEQ ID NO: 66 - protein, 442 aa, Artificial Sequence
  Synthetic Construct
EVQLLESGGGLVQPGGSLRLSCAASGFDFVNNAMIWVRKAPGKGLEWVSALSFADNTAYYATWASGRFTISRDSSKTTVYLQMNSLRAEDTAVYYCMRGDLWGPGTLVTVSSASTKGPSVFPLAPSSKSTSGGTAALGCLVKDYFPEPVTVSWNSGALTSGVHTFPAVLQSSGLYSLESVVTVPSSSLGTQTYICNVNHKPSNTKVDKKVEPKSCDKTHTCPPCPAPELLGGPSVFLFPPKPKDTLMISRTPEVTCVVVDVSHEDPEVKFNWYVDGVEVHNAKTKPREEQYGSTYRVVSVLTVLHQDWLNGKEYKCKVSNKALPAPIEKTISKAKGQPREPQVYTLPPSREEMTKNQVSLSCAVKGFYPSDIAVEWESNGQPENNYKTTPPVLDSDGSFFLVSKLTVDKSRWQQGNVFSCSVMHEALHNHYTQKSLSLSPGK

SEQ ID NO: 67 - protein, 449 aa, Artificial Sequence
  Synthetic Construct
EVQLVQSGAEVKKPGASVKVSCKASGFTFTSYYIHWVRKAPGQGLEWIGWIYPENDNTKYNEKFKDRVTITADTSTSTAYLELSSLRSEDTAVYYCARDGYSRYYFDYWGQGTLVTVSSASTKGPSVFPLAPSSKSTSGGTAALGCLVKDYFPEPVTVSWNSGALTSGVHTFPAVLQSSGLYSLESVVTVPSSSLGTQTYICNVNHKPSNTKVDKKVEPKSCDKTHTCPPCPAPELLGGPSVFLFPPKPKDTLMISRTPEVTCVVVDVSHEDPEVKFNWYVDGVEVHNAKTKPREEQYGSTYRVVSVLTVLHQDWLNGKEYKCKVSNKALPAPIEKTISKAKGQPREPQVYTLPPSREEMTKNQVSLWCLVKGFYPSDIAVEWESNGQPENNYKTTPPVLDSDGSFFLYSKLTVDKSRWQQGNVFSCSVMHEALHNHYTQKSLSLSPGK

SEQ ID NO: 68 - protein, 449 aa, Artificial Sequence
  Synthetic Construct
EVQLVQSGAEVKKPGASVKVSCKASGFTFTSYYIHWVREAPGQGLEWIGWIYPENDNTKYNEKFKDRVTITADTSTSTAYLELSSLRSEDTAVYYCARDGYSRYYFDYWGQGTLVTVSSASTKGPSVFPLAPSSKSTSGGTAALGCLVKDYFPEPVTVSWNSGALTSGVHTFPAVLQSSGLYSLKSVVTVPSSSLGTQTYICNVNHKPSNTKVDKKVEPKSCDKTHTCPPCPAPELLGGPSVFLFPPKPKDTLMISRTPEVTCVVVDVSHEDPEVKFNWYVDGVEVHNAKTKPREEQYGSTYRVVSVLTVLHQDWLNGKEYKCKVSNKALPAPIEKTISKAKGQPREPQVYTLPPSREEMTKNQVSLWCLVKGFYPSDIAVEWESNGQPENNYKTTPPVLDSDGSFFLYSKLTVDKSRWQQGNVFSCSVMHEALHNHYTQKSLSLSPGK

SEQ ID NO: 69 - protein, 449 aa, Artificial Sequence
  Synthetic Construct
EVQLVQSGAEVKKPGASVKVSCKASGFTFTSYYIHWVREAPGQGLEWIGWIYPENDNTKYNEKFKDRVTITADTSTSTAYLELSSLRSEDTAVYYCARDGYSRYYFDYWGQGTLVTVSSASTKGPSVFPLAPSSKSTSGGTAALGCLVKDYFPEPVTVSWNSGALTSGVHTFPAVLQSSGLYSLKSVVTVPSSSLGTQTYICNVNHKPSNTKVDKKVEPKSCDKTHTCPPCPAPELLGGPSVFLFPPKPKDTLMISRTPEVTCVVVDVSHEDPEVKFNWYVDGVEVHNAKTKPREEQYGSTYRVVSVLTVLHQDWLNGKEYKCKVSNKALPAPIEKTISKAKGQPREPQVYTLPPSREEMTKNQVSLSCAVKGFYPSDIAVEWESNGQPENNYKTTPPVLDSDGSFFLVSKLTVDKSRWQQGNVFSCSVMHEALHNHYTQKSLSLSPGK

SEQ ID NO: 70 - protein, 219 aa, Artificial Sequence
  Synthetic Construct
DIVMTQSPDSLAVSLGERATINCKSSQSLLNSRTRKNYLAWYQKKPGQPPKLLIYWASTRESGVPDRFSGSGSGTDFTLTISSLQAEDVAVYYCTQSFILRTFGQGTKVEIKRTVAAPSVFIFPPSDEQLKSGTASVECLLNNFYPREAKVQWKVDNALQSGNSQESVTEQDSKDSTYSLSSTLTLSKADYEKHKVYACEVTHQGLSSPVTKSFNRGEC

SEQ ID NO: 71-72 - skipped (2 entries)

SEQ ID NO: 73 - protein, 219 aa, Artificial Sequence
  Synthetic Construct
DIVMTQSPDSLAVSLGERATINCKSSQSLLNSRTRKNYLAWYQKKPGQPPKLLIYWASTRKSGVPDRFSGSGSGTDFTLTISSLQAEDVAVYYCKQSFILRTFGQGTKVEIKRTVAAPSVFIFPPSDEQLKSGTASVECLLNNFYPREAKVQWKVDNALQSGNSQESVTEQDSKDSTYSLSSTLTLSKADYEKHKVYACEVTHQGLSSPVTKSFNRGEC

SEQ ID NO: 74 - skipped

SEQ ID NO: 75 - protein, 133 aa, Artificial Sequence
  Synthetic Construct
MKPQFVGILLSSLLGAALGNRMRCYNCGGSPSSSCKEAVTTCGEGRPQPGLEQIKLPGNPPVTLIHQHPACVAAHHCNQVETESVGDVTYPAHRDCYLGDLCNSAVASHVAPAGILAAAATALTCLLPGLWSG

SEQ ID NO: 76 - DNA, 2449 bp, Artificial Sequence
  Synthetic Construct
atgaaaccccagtttgttgggatcttgctcagctccctgctaggggctgccttgggtaaggaggcggccagctagcttctcacacaggccttctgccagccggctccaccgagggcccaggtccagcgcctcttttctcctgccaggaaaccgaatgcggtgctacaactgtggtggaagccccagcagttcttgcaaagaggccgtgaccacctgtggcgagggcagaccccagccaggcctggaacagatcaagctacctggaaaccgtgagtcctcagtttctccctcttccagcagcctttccctgcctccagccccatgtcaatccttctggcttccagaaccctccaggctcagtctggctctgggcagatggtgcagctgttagaggagagcagtctgtaccccttctggctcctggcacggagcccctgagaggcccacagtccttgtgcccccacttccccacctccttattctcctaaaagaatctcataggcccattagctcacaaatgaagagctctggccctgaaaggccaaagttaaaaccaaacttcaaattttcggcattagttaaggaccagggaggggtgtgtgtgtgtgtgtgtgtgtgtgtgtgtgtgtgtgtgtacatgtttttaatattttattttaacataattttggattgacagaaaagttgcagaaatactcaacttctcctaatgctaacatcttacataaccatagcacaattatcaaaatcacaaaataactgatacaatactactaactaatctacagactttatttgatttagcaagatcctacattgcatttagctctcatgtcttcttagtctcctctgatctgtgccagttctgtttttctttgtctttcatgaccctgacacatttgaagagccctgataaattattttatacctggagtttaaaaaattacttttagggccagtgcagtcactcgcacctgtaatcccagcactttaggaggccaaggtgggaggaccacttgagcccaagagttgagaccagcctgggcaacatagggagaccctgtctctacaaaaaacaaacaaacaaacaaacaaacagattaaaaaattagttgggtgtggtggcacatgcttgtagtcctagctactcagggggctgaagagggaggatcgcttgagcctgggagattgaagctacaatgagccatgatcacgccactacactccagcctggggaacaaaatgagaccctgtctcaaaaataataataataataatttttaggctaggcttggtggcacacacttgtaatcccagcactttgggaggccaaggctgaagagtcacctgaggtcaggagtttgacaccagcctgggcagcaaagtgagacccccatctctacaaaaaatgtttttaaaaaattagccaggcatagtggcacacacctgtaatctcagtttcctgagaggctgaggcaggaggattacttgagcccaggagtttgaggctatagggaggtatgattgcaccaccacactccagcctgagtgagagagcaagatcttttctctaaaattaaataaaatcatttttagattaaacaaaaattacgtgccggatgcagtggctcacgcctgtaatcccagcactttgggaggccaaggcgggtggataacctgaggtcgggagttcaagaccagcctgatcaatgtggagaaatctcgtctctactaaaaatacaaaattagccgggtgtagtggtgcccgcctgtaataccagctactcgggaacctgaggcaggagaattgcttgaacccaagaggtggaggtcgcggtgagccgagatcacaccattgcactccagctgggcaataagagtgaaactccgtctcaaaaaaaaaaaaaaaattacagatacttgaaatactaaaaattattttatagaatgtccctcgatatttatttatctgatatttgccatgatgagattgaggtcatgcattttaagcaagaatactgcagaagtgatgttgcatccttcttgctgcatcacatcaggagtttacaaggtcaatgcattaactttgatcacttggtttcagggaggtgttttttgagggggctgaaaatccctttgggctccttgaaatcacatctgctctgccccagaaggcaagtcctgaagccaggagtccaacaccccagtttcattctctctctcagccccagtgaccttgattcaccaacatccagcctgcgtcgcagcccatcattgcaatcaagtggagacagagtcggtgggagacgtgacttatccagcccacagggactgctacctgggagacctgtgcaacagcgccgtggcaagccatgtggcccctgcaggcattttggctgcagcagctaccgccctgacctgtctcttgccaggactgtggagcggatag

SEQ ID NO: 77 - protein, 133 aa, Artificial Sequence; identical to SEQ ID NO: 75
  Synthetic Construct

SEQ ID NO: 78 - protein, 10 aa, Artificial Sequence
  Synthetic Construct
RDCYLGDLCN

SEQ ID NO: 79 - protein, 3 aa, Artificial Sequence
  Synthetic Construct
GDL

SEQ ID NO: 80 - protein, 207 aa, Artificial Sequence
  Synthetic Construct
MQSGTHWRVLGLCLLSVGVWGQDGNEEMGGITQTPYKVSISGTTVILTCPQYPGSEILWQHNDKNIGGDEDDKNIGSDEDHLSLKEFSELEQSGYYVCYPRGSKPEDANFYLYLRARVCENCMEMDVMSVATIVIVDICITGGLLLLVYYWSKNRKAKAKPVTRGAGAGGRQRGQNKERPPPVPNPDYEPIRKGQRDLYSGLNQRRI

SEQ ID NO: 81 - protein, 198 aa, Artificial Sequence
  Synthetic Construct
MQSGTRWRVLGLCLLSIGVWGQDGNEEMGSITQTPYQVSISGTTVILTCSQHLGSEAQWQHNGKNKEDSGDRLFLPEFSEMEQSGYYVCYPRGSNPEDASHHLYLKARVCENCMEMDVMAVATIVIVDICITLGLLLLVYYWSKNRKAKAKPVTRGAGAGGRQRGQNKERPPPVPNPDYEPIRKGQQDLYSGLNQRRI

SEQ ID NO: 82 - protein, 182 aa, Artificial Sequence
  Synthetic Construct
MEQGKGLAVLILAIILLQGTLAQSIKGNHLVKVYDYQEDGSVLLTCDAEAKNITWFKDGKMIGFLTEDKKKWNLGSNAKDPRGMYQCKGSQNKSKPLQVYYRMCQNCIELNAATISGFLFAEIVSIFVLAVGVYFIAGQDGVRQSRASDKQTLLPNDQLYQPLKDREDDQYSHLQGNQLRRN

SEQ ID NO: 83 - protein, 181 aa, Artificial Sequence
  Synthetic Construct
MVQGKGLTGFILAIILLQGSLAQSFEENRKLNVYNQEDGSVLLTCHVKNTNITWFKEGKMIDILTAHKNKWNLGSNTKDPRGVYQCKGSKDKSKTLQVYYRMCQNCIELNAATILGFVFAEIISIFFLAVGVYFIAGQDGVRQSRASDKQTLLPNDQLYQPLKDREDDQYSHLQGNQLRMN

SEQ ID NO: 84 - protein, 26 aa, Artificial Sequence
  Synthetic Construct
MQSGTHWRVLGLCLLSVGVWGQDGNE

SEQ ID NO: 85 - protein, 27 aa, Artificial Sequence
  Synthetic Construct
MQSGTHWRVLGLCLLSVGVWGQDGNEE

SEQ ID NO: 86 - protein, 16 aa, Artificial Sequence
  Synthetic Construct
QDGNEEMGGITQTPYK

SEQ ID NO: 87 - protein, 12 aa, Artificial Sequence
  Synthetic Construct
HRDCYLGDLCNS

SEQ ID NO: 88 - protein, 91 aa, Artificial Sequence
  Synthetic Construct
NRMRCYNCGGSPSSSCKEAVTTCGEGRPQPGLEQIKLPGNPPVTLIHQHPACVAAHHCNQVETESVGDVTYPAHRDCYLGDLCNSAGNSVT

SEQ ID NO: 89 - protein, 119 aa, Artificial Sequence
  Synthetic Construct
EVQLVQSGAEVKKPGASVKVSCKASGFTFTSYYIHWVREAPGQGLEWIGWIYPENDNTKYNEKFKDRVTITADTSTSTAYLELSSLRSEDTAVYYCARDGYSRYYFDYWGQGTLVTVSS

SEQ ID NO: 90 - protein, 112 aa, Artificial Sequence
  Synthetic Construct
DIVMTQSPDSLAVSLGERATINCKSSQSLLNSRTRKNYLAWYQKKPGQPPKLLIYWASTRESGVPDRFSGSGSGTDFTLTISSLQAEDVAVYYCTQSFILRTFGQGTKVEIK

SEQ ID NO: 91 - skipped

SEQ ID NO: 92 - protein, 112 aa, Artificial Sequence
  Synthetic Construct
DIVMTQSPDSLAVSLGERATINCKSSQSLLNSRTRKNYLAWYQKKPGQPPKLLIYWASTRKSGVPDRFSGSGSGTDFTLTISSLQAEDVAVYYCKQSFILRTFGQGTKVEIK

SEQ ID NO: 93 - protein, 112 aa, Artificial Sequence
  Synthetic Construct
DIVMTQSPDSLAVSLGERATINCKSSQSLLNSRTRKNYLAWYQQKPGQSPKLLIYWTSTRKSGVPDRFSGSGSGTDFTLTISSLQAEDVAVYYCKQSFILRTFGQGTKVEIK

SEQ ID NO: 94 - protein, 112 aa, Artificial Sequence
  Synthetic Construct
DIVMTQSPDSLAVSLGERATINCKSSQSLLNSRTRKNYLAWYQQKPGQPPKLLIYWASTRKSGVPDRFSGSGSGTDFTLTISSLQAEDVAVYYCKQSFILRTFGQGTKVEIK

SEQ ID NO: 95 - protein, 222 aa, Artificial Sequence
  Synthetic Construct
EVQLVQSGAEVKKPGASVKVSCKASGYTFTTYVMHWVRQAPGQGLEWMGYINPYNDGTKYNEKFKGRVTMTRDTSISTAYMELSRLRSDDTAVYYCGRRNFDYWGQGTLVTVSSASTKGPSVFPLAPSSKSTSGGTAALGCLVKDYFPEPVTVSWNSGALTSGVHTFPAVLQSSGLYSLSSVVTVPSSSLGTQTYICNVNHKPSNTKVDKKVEPKSCDKTHT

SEQ ID NO: 96 - protein, 216 aa, Artificial Sequence
  Synthetic Construct
EVQLLESGGGLVQPGGSLRLSCAASGFDFVNNAMIWVRQAPGKGLEWVSALSFADNTAYYATWASGRFTISRDSSKTTVYLQMNSLRAEDTAVYYCMRGDLWGPGTLVTVSSASTKGPSVFPLAPSSKSTSGGTAALGCLVKDYFPEPVTVSWNSGALTSGVHTFPAVLQSSGLYSLSSVVTVPSSSLGTQTYICNVNHKPSNTKVDKKVEPKSCD

SEQ ID NO: 97 - protein, 218 aa, Artificial Sequence
  Synthetic Construct
DIQMTQSPSTLSASVGDRVTITCQASESITRYLNWYQQKPGKAPKLLIYDASKLPSGVPSRFSGSGSGTEFTLTISSLQPDDFATYYCQSTSFRGRSYQNTFGGGTKVEIKRTVAAPSVFIFPPSDEQLKSGTASVVCLLNNFYPREAKVQWKVDNALQSGNSQESVTEQDSKDSTYSLSSTLTLSKADYEKHKVYACEVTHQGLSSPVTKSFNRGEC

SEQ ID NO: 98 - protein, 119 aa, Artificial Sequence
  Synthetic Construct
EVQLVQSGAEVKKPGASVKVSCKASGYTFTNYYIHWVRQAPGQGLEWIGWIYPGDGNTKYNEKFKGRATLTADTSTSTAYLELSSLRSEDTAVYYCARDSYSNYYFDYWGQGTLVTVSS

SEQ ID NO: 99 - protein, 13 aa, Artificial Sequence
  Synthetic Construct
QSTSFRGRSYNNT

SEQ ID NO: 100 - protein, 13 aa, Artificial Sequence
  Synthetic Construct
QSTSFRGRSYQNV

SEQ ID NO: 101 - protein, 13 aa, Artificial Sequence
  Synthetic Construct
QSTSFRGRSYSNT

SEQ ID NO: 102 - protein, 13 aa, Artificial Sequence
  Synthetic Construct
QSTSFRGRSYSNA

SEQ ID NO: 103 - protein, 13 aa, Artificial Sequence
  Synthetic Construct
QSTSFRGRSYANT

SEQ ID NO: 104 - protein, 13 aa, Artificial Sequence
  Synthetic Construct
QSTSFRGRSYNNA

SEQ ID NO: 105 - protein, 13 aa, Artificial Sequence
  Synthetic Construct
QSTSFRGRSYNNV

SEQ ID NO: 106 - protein, 13 aa, Artificial Sequence
  Synthetic Construct
QSTSFRGRSYGNT

SEQ ID NO: 107 - protein, 13 aa, Artificial Sequence
  Synthetic Construct
QSTSFRGRSYSNV

SEQ ID NO: 108 - protein, 112 aa, Artificial Sequence
  Synthetic Construct
DIVMTQSPDSLAVSLGERATINCKSSQSLLNSRTRKNYLAWYQKKPGQSPKLLIYWTSTRKSGVPDRFSGSGSGTDFTLTISSLQAEDVAVYYCKQSFILRTFGQGTKVEIK

SEQ ID NO: 109 - protein, 119 aa, Artificial Sequence
  Synthetic Construct
EVQLVQSGAEVKKPGASVKVSCKASGYTFTNYYIHWVRKAPGQGLEWIGWIYPGDGNTKYNEKFKGRATLTADTSTSTAYLELSSLRSEDTAVYYCARDSYSNYYFDYWGQGTLVTVSS

SEQ ID NO: 110 - protein, 7 aa, Artificial Sequence
  Synthetic Construct
WASTRIS

SEQ ID NO: 111 - protein, 5 aa, Artificial Sequence
  Synthetic Construct
NNAMS

SEQ ID NO: 112 - protein, 17 aa, Artificial Sequence
  Synthetic Construct
SLSFADNTAYYATWASG

SEQ ID NO: 113 - protein, 17 aa, Artificial Sequence
  Synthetic Construct
ILSFADNTAYYATWASG

SEQ ID NO: 114 - protein, 442 aa, Artificial Sequence
  Synthetic Construct
EVQLLESGGGLVQPGGSLRLSCAASGFDFVNNAMIWVRQAPGKGLEWVSALSFADNTAYYATWASGRFTISRDSSKTTVYLQMNSLRAEDTAVYYCMRGDLWGPGTLVTVSSASTKGPSVFPLAPSSKSTSGGTAALGCLVKDYFPEPVTVSWNSGALTSGVHTFPAVLQSSGLYSLSSVVTVPSSSLGTQTYICNVNHKPSNTKVDKKVEPKSCDKTHTCPPCPAPELLGGPSVFLFPPKPKDTLMISRTPEVTCVVVDVSHEDPEVKFNWYVDGVEVHNAKTKPREEQYGSTYRVVSVLTVLHQDWLNGKEYKCKVSNKALPAPIEKTISKAKGQPREPQVYTLPPSREEMTKNQVSLWCLVKGFYPSDIAVEWESNGQPENNYKTTPPVLDSDGSFFLYSKLTVDKSRWQQGNVFSCSVMHEALHNHYTQKSLSLSPGK

SEQ ID NO: 115 - protein, 218 aa, Artificial Sequence; identical to SEQ ID NO: 97
  Synthetic Construct

SEQ ID NO: 116 - protein, 7 aa, Artificial Sequence
  Synthetic Construct
GRSYNNT

SEQ ID NO: 117 - protein, 111 aa, Artificial Sequence
  Synthetic Construct
DIQMTQSPSSLSASVGDRVTITCQASESITRYLNWYQQKPGKPPKLLIYDASKLPSGVPSRFSGSGSGTDFTLTISSLQPEDFATYYCQSTSFRGRSYNNTFGGGTKVEIK

SEQ ID NO: 118 - protein, 111 aa, Artificial Sequence
  Synthetic Construct
DIQMTQSPSTLSASVGDRVTITCQASESITRYLNWYQQKPGKPPKLLIYDASKLPSGVPSRFSGSGSGTEFTLTISSLQPDDFATYYCQSTSFRGRSYNNTFGGGTKVEIK

SEQ ID NO: 119 - protein, 111 aa, Artificial Sequence
  Synthetic Construct
DIVMTQSPDSLAVSLGERATINCQASESITRYLNWYQQKPGQPPKLLIYDASKLPSGVPDRFSGSGSGTDFTLTISSLQAEDVAVYYCQSTSFRGRSYNNTFGGGTKVEIK

SEQ ID NO: 120 - protein, 112 aa, Artificial Sequence
  Synthetic Construct
EQQLLESGGGLVQPGGSLRLSCAASGFDFVNNAMSWVRQAPGKGLEWIAALSFADNTAYYATWASGRFTISKDSSKTTVYLQMNSLRAEDTAVYFCMRGDLWGPGTLVTVSS

SEQ ID NO: 121 - protein, 112 aa, Artificial Sequence
  Synthetic Construct
EQQLVESGGGVVQPGRSLRLSCAASGFDFVNNAMSWVRQAPGKGLEWIAALSFADNTAYYATWASGRFTISKDSSKNTVYLQMNSLRAEDTAVYFCMRGDLWGPGTLVTVSS

SEQ ID NO: 122 - protein, 111 aa, Artificial Sequence
  Synthetic Construct
DIQMTQSPSTLSASVGDRVTITCQASESITRYLNWYQQKPGKPPKLLIYDASKLPSGVPSRFSGSGSGTEFTLTISSLQPDDFATYYCQSTSFRGRSYQNTFGGGTKVEIK

SEQ ID NO: 123 - protein, 112 aa, Artificial Sequence
  Synthetic Construct
EQQLVESGGGVVQPGRSLRLSCAASGFDFVNNAMIWVRQAPGKGLEWIAALSFADNTAYYATWASGRFTISKDSSKNTVYLQMNSLRAEDTAVYFCMRGDLWGPGTLVTVSS

SEQ ID NO: 124 - protein, 107 aa, Artificial Sequence
  Synthetic Construct
DIQMTQSPSTLSASVGDRVTITCRASQSISSWLAWYQQKPGKAPKLLIYDASSLESGVPSRFSGSGSGTEFTLTISSLQPDDFATYYCQQYNSYSLTFGGGTKVEIK

SEQ ID NO: 125 - protein, 112 aa, Artificial Sequence
  Synthetic Construct
EVQLLESGGGLVQPGGSLRLSCAASGFTFSSYAMSWVRQAPGKGLEWVSAISGSGGSTYYADSVKGRFTISRDNSKNTLYLQMNSLRAEDTAVYYCAKFDLWGRGTLVTVSS

SEQ ID NO: 126 - protein, 112 aa, Artificial Sequence
  Synthetic Construct
DIVMTQSPDSLAVSLGERATINCKSSQSLLNSRTRKNYLAWYQEKPGQSPKLLIYWTSTRKSGVPDRFSGSGSGTDFTLTISSLQAEDVAVYYCKQSFILRTFGQGTKVEIK

SEQ ID NO: 127 - protein, 119 aa, Artificial Sequence
  Synthetic Construct
EVQLVQSGAEVKKPGASVKVSCKASGYTFTNYYIHWVREAPGQGLEWIGWIYPGDGNTKYNEKFKGRATLTADTSTSTAYLELSSLRSEDTAVYYCARDSYSNYYFDYWGQGTLVTVSS

SEQ ID NO: 128 - protein, 112 aa, Artificial Sequence
  Synthetic Construct
DIVMTQSPDSLAVSLGERATINCKSSQSLLNSRTRKNYLAWYQQKPGQPPKLLIYWTSTRKSGVPDRFSGSGSGTDFTLTISSLQAEDVAVYYCKQSFILRTFGQGTKVEIK

SEQ ID NO: 129 - protein, 112 aa, Artificial Sequence
  Synthetic Construct
DIVMTQSPDSLAVSLGERATINCKSSQSLLNSRTRKNYLAWYQQKPGQSPKLLIYWASTREKGVPDRFSGSGSGTDFTLTISSLQAEDVAVYYCKQSFILRTFGQGTKVEIK

SEQ ID NO: 130 - protein, 111 aa, Artificial Sequence
  Synthetic Construct
DIVMTQTPSSVSAAVGGTVTINCQASESITRYLNWYQQKPGQPPKLLIYDASKLPSGVPSRFKGSGSGTQFTLTTSDLECADAATYYCQSTSFRGRSYNNTFGGGTEVVVK

SEQ ID NO: 131 - protein, 111 aa, Artificial Sequence
  Synthetic Construct
QQQLEESGGDLVKPGASLTLTCTASGFDFVNNAMCWVRQAPGKGLEWIACLSFADNTAYYATWASGRFTISKISSTTVTLRMTSLTGADTATYFCMRGDLWGPGTLVTVSS

SEQ ID NO: 132 - protein, 111 aa, Artificial Sequence
  Synthetic Construct
EAVLTQSPGTLSLSPGERATLSCQSSESVWHNNWLAWFQQKPGQRPRLLIYGASTLASGVPDRFSGSGSGTDFTLTISRLEPEDFAVYYCAGGYSSSDAHVFGGGTKVEIK

SEQ ID NO: 133 - protein, 111 aa, Artificial Sequence
  Synthetic Construct
DAQLTQSPSTLSASVGDRVTITCQSSESVWHNNWLAWFQQKPGKRPKLLIYGASTLASGVPSRFSGSGSGTEFTLTISSLQPDDFATYYCAGGYSSSDAHVFGGGTKVEIK

SEQ ID NO: 134 - protein, 111 aa, Artificial Sequence
  Synthetic Construct
DAVLTQSPDSLAVSLGERATINCQSSESVWHNNWLAWFQQKPGQRPKLLIYGASTLASGVPDRFSGSGSGTDFTLTISSLQAEDVAVYYCAGGYSSSDAHVFGGGTKVEIK

SEQ ID NO: 135 - protein, 118 aa, Artificial Sequence
  Synthetic Construct
EQQLVESGGGLIQPGGSLRLSCAVSGLSLSTNSINWVRQAPGKGLEWIGYIYHGDGIADYASWAKGRFTISKDSSKNTVYLQMNSLRAEDTAVYFCASGAGYSLFTLWGPGTLVTVSS

SEQ ID NO: 136 - protein, 118 aa, Artificial Sequence
  Synthetic Construct
EQQLQESGPGLVKPPGTLSLTCAVSGLSLSTNSINWVRQPPGKGLEWIGYIYHGDGIADYASWAKGRFTISKDSSKTQVSLKLSSVTAADTAVYFCASGAGYSLFTLWGPGTLVTVSS

SEQ ID NO: 137 - protein, 118 aa, Artificial Sequence
  Synthetic Construct
EQQLVESGGGLVQPGGSLRLSCAVSGLSLSTNSINWVRQAPGKGLEWIGYIYHGDGIADYASWAKGRFTISKDSAKNSVYLQMNSLRAEDTAVYFCASGAGYSLFTLWGPGTLVTVSS

SEQ ID NO: 138 - protein, 111 aa, Artificial Sequence
  Synthetic Construct
AAVLTQTPSPVSAAVGGTITINCQSSESVWHNNWLAWFQQKPGQRPRLLIYGASTLASGVPSRFSGTGSGTQFTLTISDVQCDDAATYYCAGGYSSSDAHVFGRGTAVVVK

SEQ ID NO: 139 - protein, 111 aa, Artificial Sequence
  Synthetic Construct
DAQMTQSPSTLSASVGDRVTITCQSSESVWHNNWLAWFQQKPGKRPKLLIYGASTLASGVPSRFSGSGSGTEFTLTISSLQPDDFATYYCAGGYSSSDAHVFGGGTKVEIK

SEQ ID NO: 140 - protein, 111 aa, Artificial Sequence
  Synthetic Construct
EAVLTQSPGTLSLSPGERATLSCQSSESVWHNNWLAWFQQKPGQAPRLLIYGASTLASGVPDRFSGSGSGTDFTLTISRLEPEDFAVYYCAGGYSSSDAHVFGGGTKVEIK

SEQ ID NO: 141 - protein, 116 aa, Artificial Sequence
  Synthetic Construct
QSLEESGGGLVKPGGTLTLTCTVSGLSLSTNSINWVRQAPGKGLEWIGYIYHGDGIADYASWAKGRFTISKTSSTTVTLRMTSLTVADTATYFCASGAGYSLFTLWGPGTLVTVSS

SEQ ID NO: 142 - protein, 118 aa, Artificial Sequence
  Synthetic Construct
EVQLVESGGGLVQPGGSLRLSCAASGLSLSTNSINWVRQAPGKGLEWVSYIYHGDGIADYASWAKGRFTISRDNAKNSLYLQMNSLRAEDTAVYYCASGAGYSLFTLWGRGTLVTVSS

SEQ ID NO: 143 - protein, 118 aa, Artificial Sequence
  Synthetic Construct
EVQLVESGGGLIQPGGSLRLSCAASGLSLSTNSINWVRQAPGKGLEWVSYIYHGDGIADYASWAKGRFTISRDNSKNTLYLQMNSLRAEDTAVYYCASGAGYSLFTLWGRGTLVTVSS

SEQ ID NO: 144 - protein, 108 aa, Artificial Sequence
  Synthetic Construct
EIVLTQSPGTLSLSPGERATLSCRASQSVSSSYLAWYQQKPGQAPRLLIYGASSRATGIPDRFSGSGSGTDFTLTISRLEPEDFAVYYCQQYGSSPLTFGGGTKVEIK

SEQ ID NO: 145 - protein, 111 aa, Artificial Sequence
  Synthetic Construct
EVQLVESGGGLIQPGGSLRLSCAASGFTVSSNYMSWVRQAPGKGLEWVSVIYSGGSTYYADSVKGRFTISRDNSKNTLYLQMNSLRAEDTAVYYCARFDLWGRGTLVTVSS

SEQ ID NO: 146 - protein, 112 aa, Artificial Sequence
  Synthetic Construct
EVQLVESGGGLVQPGGSLRLSCAASGFTFSSYSMNWVRQAPGKGLEWVSYISSSSSTIYYADSVKGRFTISRDNAKNSLYLQMNSLRAEDTAVYYCARFDLWGRGTLVTVSS

SEQ ID NO: 147 - protein, 220 aa, Artificial Sequence
  Synthetic Construct
DIVMTQSPDSLAVSLGERATINCKSSQSLLLSGNQENYLAWHQQKPGQPPKTLITWASTRISGVPDRFSGSGSGTDFTLTISSLQAEDVAVYYCQQSYSAPYTFGGGTKVEIKRTVAAPSVFIFPPSDEQLKSGTASVVCLLNNFYPREAKVQWKVDNALQSGNSQESVTEQDSKDSTYSLSSTLTLSKADYEKHKVYACEVTHQGLSSPVTKSFNRGEC